European Patent Specification EP 4 172 199 B1, published May 14, 2025. Title: ALPHA-SYNUCLEIN PROTOFIBRIL-BINDING ANTIBODIES. Applicant: BioArctic AB. The sequence listing filed with the application follows.

SEQUENCE LISTING (20 sequences)

SEQ ID NO: 1 - protein, 118 aa, artificial
  BAN0805 VH
QVQLQESGPGLVKPSETLSLTCTVSGFSLTSYGVHWIRQPPGKGLEWIGVIWRGGSTDYSAAFMSRLTISKDTSKNQVSLKLSSVTAADTAVYYCAKLLRSVGGFADWGQGTMVTVSS

SEQ ID NO: 2 - protein, 112 aa, artificial
  BAN0805 VL
DIVMTQSPLSLPVTPGEPASISCRSSQTIVHNNGNTYLEWYLQKPGQSPQLLIYKVSNRFSGVPDRFSGSGSGTDFTLKISRVEAEDVGVYYCFQGSHVPFTFGQGTKLEIK

SEQ ID NO: 3 - protein, 444 aa, artificial
  BAN0805 Heavy Chain
QVQLQESGPGLVKPSETLSLTCTVSGFSLTSYGVHWIRQPPGKGLEWIGVIWRGGSTDYSAAFMSRLTISKDTSKNQVSLKLSSVTAADTAVYYCAKLLRSVGGFADWGQGTMVTVSSASTKGPSVFPLAPCSRSTSESTAALGCLVKDYFPEPVTVSWNSGALTSGVHTFPAVLQSSGLYSLSSVVTVPSSSLGTKTYTCNVDHKPSNTKVDKRVESKYGPPCPPCPAPEFLGGPSVFLFPPKPKDTLMISRTPEVTCVVVDVSQEDPEVQFNWYVDGVEVHNAKTKPREEQFNSTYRVVSVLTVLHQDWLNGKEYKCKVSNKGLPSSIEKTISKAKGQPREPQVYTLPPSQEEMTKNQVSLTCLVKGFYPSDIAVEWESNGQPENNYKTTPPVLDSDGSFFLYSRLTVDKSRWQEGNVFSCSVMHEALHNHYTQKSLSLSLG

SEQ ID NO: 4 - protein, 219 aa, artificial
  BAN0805 Light Chain
DIVMTQSPLSLPVTPGEPASISCRSSQTIVHNNGNTYLEWYLQKPGQSPQLLIYKVSNRFSGVPDRFSGSGSGTDFTLKISRVEAEDVGVYYCFQGSHVPFTFGQGTKLEIKRTVAAPSVFIFPPSDEQLKSGTASVVCLLNNFYPREAKVQWKVDNALQSGNSQESVTEQDSKDSTYSLSSTLTLSKADYEKHKVYACEVTHQGLSSPVTKSFNRGEC

SEQ ID NO: 5 - protein, 10 aa, artificial
  BAN0805 VH-CDR-1 (Chothia)
GFSLTSYGVH

SEQ ID NO: 6 - protein, 14 aa, artificial
  BAN0805 VH-CDR-2 (Chothia)
VIWRGGSTDYSAAF

SEQ ID NO: 7 - protein, 10 aa, artificial
  BAN0805 VH-CDR-3 (Kabat/Chothia)
LLRSVGGFAD

SEQ ID NO: 8 - protein, 16 aa, artificial
  BAN0805 VL-CDR-1 (Kabat/Chothia)
RSSQTIVHNNGNTYLE

SEQ ID NO: 9 - protein, 7 aa, artificial
  BAN0805 VL-CDR-2 (Kabat/Chothia)
KVSNRFS

SEQ ID NO: 10 - protein, 9 aa, artificial
  BAN0805 VL-CDR-3 (Kabat/Chothia)
FQGSHVPFT

SEQ ID NO: 11 - DNA, 1395 bp, artificial
  BAN0805 HC gene with signal sequence
atggaatggtcctgggtgttcctgttcttcctgtccgtgaccaccggcgtgcactctcaggttcagctgcaagagtctggccctggcctggtcaagccttccgaaacactgtctctgacctgcaccgtgtccggcttctccctgacatcttatggggtgcactggatcagacagcctccaggcaaaggcctggaatggatcggagtgatttggagaggcggctccaccgattactccgccgccttcatgtcccggctgaccatctctaaggacacctccaagaaccaggtgtccctgaagctgtcctctgtgaccgctgctgataccgccgtgtactactgtgccaagctgctgagatctgtcggcggctttgctgattggggccagggcacaatggtcaccgtgtctagcgcttctacaaagggcccaagcgtgttccccctggccccctgctccagaagcaccagcgagagcacagccgccctgggctgcctggtgaaggactacttccccgagcccgtgaccgtgtcctggaacagcggagccctgaccagcggcgtgcacaccttccccgccgtgctgcagagcagcggcctgtacagcctgagcagcgtggtgaccgtgcccagcagcagcctgggcaccaagacctacacctgtaacgtggaccacaagcccagcaacaccaaggtggacaagagggtggagagcaagtacggcccaccctgccccccctgcccagcccccgagttcctgggcggacccagcgtgttcctgttcccccccaagcccaaggacaccctgatgatcagcagaacccccgaggtgacctgtgtggtggtggacgtgtcccaggaggaccccgaggtccagttcaactggtacgtggacggcgtggaggtgcacaacgccaagaccaagcccagagaggagcagtttaacagcacctaccgggtggtgtccgtgctgaccgtgctgcaccaggactggctgaacggcaaagagtacaagtgtaaggtctccaacaagggcctgccaagcagcatcgaaaagaccatcagcaaggccaagggccagcctagagagccccaggtctacaccctgccacccagccaagaggagatgaccaagaaccaggtgtccctgacctgtctggtgaagggcttctacccaagcgacatcgccgtggagtgggagagcaacggccagcccgagaacaactacaagaccacccccccagtgctggacagcgacggcagcttcttcctgtacagcaggctgaccgtggacaagtccagatggcaggagggcaacgtctttagctgctccgtgatgcacgaggccctgcacaaccactacacccagaagagcctgagcctgtccctgggctgatga

SEQ ID NO: 12 - DNA, 723 bp, artificial
  BAN0805 LC gene with signal sequence
atgtctgtgcctacacaggttctgggactgctgctgctgtggctgaccgacgccagatgcgacatcgtgatgacccagtctccactgagcctgcctgtgacacctggcgagcctgcttccatctcctgcagatcctctcagaccatcgtgcacaacaacggcaacacctacctggaatggtatctgcagaagcccggccagtctcctcagctgctgatctacaaggtgtccaaccggttctctggcgtgcccgacagattttccggctctggctctggcaccgacttcaccctgaagatctccagagtggaagccgaggacgtgggcgtgtactactgcttccaaggctctcacgtgcccttcacctttggccagggcaccaagctggaaatcaagcgtacggtggccgctcccagcgtgttcatcttccccccaagcgacgagcagctgaagagcggcaccgccagcgtggtgtgtctgctgaacaacttctaccccagggaggccaaggtgcagtggaaggtggacaacgccctgcagagcggcaacagccaggagagcgtcaccgagcaggacagcaaggactccacctacagcctgagcagcaccctgaccctgagcaaggccgactacgagaagcacaaggtgtacgcctgtgaggtgacccaccagggcctgtccagccccgtgaccaagagcttcaacaggggcgagtgctgatga

SEQ ID NO: 13 - DNA, 413 bp, artificial
  BAN0805 VH gene with signal sequence
atggaatggtcctgggtgttcctgttcttcctgtccgtgaccaccggcgtgcactctcaggttcagctgcaagagtctggccctggcctggtcaagccttccgaaacactgtctctgacctgcaccgtgtccggcttctccctgacatcttatggggtgcactggatcagacagcctccaggcaaaggcctggaatggatcggagtgatttggagaggcggctccaccgattactccgccgccttcatgtcccggctgaccatctctaaggacacctccaagaaccaggtgtccctgaagctgtcctctgtgaccgctgctgataccgccgtgtactactgtgccaagctgctgagatctgtcggcggctttgctgattggggccagggcacaatggtcaccgtgtctagcgc

SEQ ID NO: 14 - DNA, 396 bp, artificial
  BAN0805 VL gene with signal sequence
atgtctgtgcctacacaggttctgggactgctgctgctgtggctgaccgacgccagatgcgacatcgtgatgacccagtctccactgagcctgcctgtgacacctggcgagcctgcttccatctcctgcagatcctctcagaccatcgtgcacaacaacggcaacacctacctggaatggtatctgcagaagcccggccagtctcctcagctgctgatctacaaggtgtccaaccggttctctggcgtgcccgacagattttccggctctggctctggcaccgacttcaccctgaagatctccagagtggaagccgaggacgtgggcgtgtactactgcttccaaggctctcacgtgcccttcacctttggccagggcaccaagctggaaatcaag

SEQ ID NO: 15 - protein, 5 aa, artificial
  BAN0805 VH-CDR-1 (Kabat)
SYGVH

SEQ ID NO: 16 - protein, 16 aa, artificial
  BAN0805 VH-CDR-2 (Kabat)
VIWRGGSTDYSAAFMS

SEQ ID NO: 17 - DNA, 1335 bp, artificial
  BAN0805 HC gene
caggttcagctgcaagagtctggccctggcctggtcaagccttccgaaacactgtctctgacctgcaccgtgtccggcttctccctgacatcttatggggtgcactggatcagacagcctccaggcaaaggcctggaatggatcggagtgatttggagaggcggctccaccgattactccgccgccttcatgtcccggctgaccatctctaaggacacctccaagaaccaggtgtccctgaagctgtcctctgtgaccgctgctgataccgccgtgtactactgtgccaagctgctgagatctgtcggcggctttgctgattggggccagggcacaatggtcaccgtgtctagcgcttctacaaagggcccaagcgtgttccccctggccccctgctccagaagcaccagcgagagcacagccgccctgggctgcctggtgaaggactacttccccgagcccgtgaccgtgtcctggaacagcggagccctgaccagcggcgtgcacaccttccccgccgtgctgcagagcagcggcctgtacagcctgagcagcgtggtgaccgtgcccagcagcagcctgggcaccaagacctacacctgtaacgtggaccacaagcccagcaacaccaaggtggacaagagggtggagagcaagtacggcccaccctgccccccctgcccagcccccgagttcctgggcggacccagcgtgttcctgttcccccccaagcccaaggacaccctgatgatcagcagaacccccgaggtgacctgtgtggtggtggacgtgtcccaggaggaccccgaggtccagttcaactggtacgtggacggcgtggaggtgcacaacgccaagaccaagcccagagaggagcagtttaacagcacctaccgggtggtgtccgtgctgaccgtgctgcaccaggactggctgaacggcaaagagtacaagtgtaaggtctccaacaagggcctgccaagcagcatcgaaaagaccatcagcaaggccaagggccagcctagagagccccaggtctacaccctgccacccagccaagaggagatgaccaagaaccaggtgtccctgacctgtctggtgaagggcttctacccaagcgacatcgccgtggagtgggagagcaacggccagcccgagaacaactacaagaccacccccccagtgctggacagcgacggcagcttcttcctgtacagcaggctgaccgtggacaagtccagatggcaggagggcaacgtctttagctgctccgtgatgcacgaggccctgcacaaccactacacccagaagagcctgagcctgtccctgggctga

SEQ ID NO: 18 - DNA, 660 bp, artificial
  BAN0805 LC gene
gacatcgtgatgacccagtctccactgagcctgcctgtgacacctggcgagcctgcttccatctcctgcagatcctctcagaccatcgtgcacaacaacggcaacacctacctggaatggtatctgcagaagcccggccagtctcctcagctgctgatctacaaggtgtccaaccggttctctggcgtgcccgacagattttccggctctggctctggcaccgacttcaccctgaagatctccagagtggaagccgaggacgtgggcgtgtactactgcttccaaggctctcacgtgcccttcacctttggccagggcaccaagctggaaatcaagcgtacggtggccgctcccagcgtgttcatcttccccccaagcgacgagcagctgaagagcggcaccgccagcgtggtgtgtctgctgaacaacttctaccccagggaggccaaggtgcagtggaaggtggacaacgccctgcagagcggcaacagccaggagagcgtcaccgagcaggacagcaaggactccacctacagcctgagcagcaccctgaccctgagcaaggccgactacgagaagcacaaggtgtacgcctgtgaggtgacccaccagggcctgtccagccccgtgaccaagagcttcaacaggggcgagtgctga

SEQ ID NO: 19 - DNA, 356 bp, artificial
  BAN0805 VH gene
caggttcagctgcaagagtctggccctggcctggtcaagccttccgaaacactgtctctgacctgcaccgtgtccggcttctccctgacatcttatggggtgcactggatcagacagcctccaggcaaaggcctggaatggatcggagtgatttggagaggcggctccaccgattactccgccgccttcatgtcccggctgaccatctctaaggacacctccaagaaccaggtgtccctgaagctgtcctctgtgaccgctgctgataccgccgtgtactactgtgccaagctgctgagatctgtcggcggctttgctgattggggccagggcacaatggtcaccgtgtctagcgc

SEQ ID NO: 20 - DNA, 336 bp, artificial
  BAN0805 VL gene
gacatcgtgatgacccagtctccactgagcctgcctgtgacacctggcgagcctgcttccatctcctgcagatcctctcagaccatcgtgcacaacaacggcaacacctacctggaatggtatctgcagaagcccggccagtctcctcagctgctgatctacaaggtgtccaaccggttctctggcgtgcccgacagattttccggctctggctctggcaccgacttcaccctgaagatctccagagtggaagccgaggacgtgggcgtgtactactgcttccaaggctctcacgtgcccttcacctttggccagggcaccaagctggaaatcaag